European Patent Application EP 4 567 124 A1, published June 11, 2025. Title: Biocatalytic process for the production of 4-hydroxymethylfurfural. Applicant: CASCAT GmbH. The sequence listing filed with the application follows.

SEQUENCE LISTING (70 sequences)

SEQ ID NO: 1 - protein, 475 aa, Bacillus flavocaldarius KP1228
MAWYEGAFFYQIFPDRFFRAGPPGRPAPAGPFEPWEDPPTLRGFKGGTLWGVAEKLPYLLDLGVEAIYLNPVFASTANHRYHTVDYFQVDPILGGNEALRYLLEVAHAHGVRVILDGVFNHTGRGFFAFQHLMENGEQSPYRDWYHVKGFPLKAYTAHPNYEAWWGNPELPKLKVETPAVREYLLAVAEHWIRFGVDGWRLDVPNEIPDPTFWREFRQRVKGANPEAYIVGEIWEEADFWLQGDMFDAVMNYPLARAVLGFVGGEALDRDLAAQTGLGRIEPLQALAFSHRLEDLFGRYRPEVVRAQMNLLTSHDTPRLLSLMRGSVERARLALALLFLLPGNPTVYYGEEVGMAGGKDPENRGGMVWEEARWQKDLRETVKRLARLRKEHPALRTAPYLRIYAQDGHLAFARGPYLVVVNASPHPFRQDFPLHGVFPRGGRAVDLLSGEVCTPQGGRLCGPVLPPFSLALWREA

SEQ ID NO: 2 - DNA, 1428 bp, Bacillus flavocaldarius KP1228
  source 1..1428: mol_type = other DNA
atggcatggtatgaaggtgcctttttctatcagatttttccggatcgtttttttcgtgcaggtccgcctggtcgtccggcaccggcaggtccgtttgaaccgtgggaagatccgcctacactgcgtggttttaaaggtggcaccctgtggggtgttgcagaaaaactgccgtatctgctggatctgggtgttgaagcaatttatctgaatccggtttttgcaagcaccgccaatcatcgttatcataccgttgattattttcaggtggacccgattcttggtggtaatgaagcactgcgttacctgctggaagttgcacatgcacatggtgttcgtgttattctggatggtgtttttaatcataccggtcgtggtttttttgcctttcagcatctgatggaaaatggtgaacagagcccgtatcgtgattggtatcatgttaaaggttttccgctgaaagcatataccgcacatccgaattatgaagcatggtggggtaatccggaactgccgaaactgaaagttgaaacaccggcagttcgtgaatatttactggcagttgcagaacattggattcgttttggtgttgatggttggcgtctggatgttccgaatgaaattcctgatccgaccttttggcgtgaatttcgtcagcgtgtgaaaggtgcaaatccggaagcatatattgttggcgaaatttgggaagaagcagatttttggctgcagggtgatatgtttgatgccgttatgaattatccgctggcacgtgcagttctgggttttgttggtggtgaagccctggatcgtgatctggcagcacagacaggtctgggtcgtattgaaccgctgcaggcactggcatttagccatcgtctggaagatttatttggtcgttatcgtccggaagttgttcgtgcacagatgaatctgctgaccagccatgatacaccgcgtctgctgagcctgatgcgtggtagcgttgaacgtgcccgtctggcactggccctgctgtttctgctgcctggtaatccgaccgtttattatggtgaagaggttggtatggcaggcggtaaagatcctgaaaatcgtggtggtatggtgtgggaagaagcccgttggcagaaagatctgcgtgaaaccgttaaacgcctggcacgtctgcgtaaagaacatccggcactgcgtaccgcaccttatctgcgtatttatgcacaggatggtcatctggcatttgcacgtggtccgtatctggttgttgttaatgcaagtccgcatccgtttcgtcaggattttcctctgcatggtgtgtttccgcgtggtggtcgtgcagttgatctgctgagtggtgaagtttgtacaccgcaaggtggtcgtctgtgtggtccggttctgcctccgtttagcctggcactgtggcgtgaagcataa

SEQ ID NO: 3 - protein, 501 aa, Meiothermus ruber
MQLQRAFGILLHPTSFPGRWGIGALGREAERFLDWLADAGARWWQVLPLGPTSYGDSPYQSFSAFAGNPYLVDPEMLIEKGWLEQSEAPPPYPTQRVDYGWLYQTRWPLLRRAFAGFRARASAQDKTRLEAFIEAERFWLEDYALFMALKTRFDGKPWNEWSPELRDREPAALARAREELAEEVALYEWIQWLFYLEWGQTKAYAESKGIQIIGDMPIFVAFDSSDVWANPQYFYLEADGNPTVVAGVPPDYFSETGQLWGNPLYRWDVMERDNFAWWIARIRQSLKQCHLVRIDHFRGFEAYWEVPFGRPNAVEGRWVKAPGEKLFAAVRAQLSDAPIIAEDLGVITPEVEALRDGFGFPGMKILQFAFSGEDNAFLPHNYPAHGNVVVYSGTHDNDTTLGWFRTAPEAERAFMRAYLARYGIRCLSEYEVAGALIELAFKSPAKLAIVPLQDVLGLGPEARMNFPGRLGDNWAWRYAEGDLEPGLAAGLRALAEASQRA

SEQ ID NO: 4 - DNA, 1506 bp, Meiothermus ruber
  source 1..1506: mol_type = genomic DNA
atgcaactccaacgcgcttttggaattttgctccaccccaccagttttccgggtcgctgggggattggggctctgggccgcgaggccgagcggtttttggactggctggccgatgcgggagcccgctggtggcaggtcttaccgctgggccctaccagttacggcgactcgccgtaccagtccttctcggcttttgccggtaacccgtatttggttgaccccgagatgctgattgaaaaaggctggctggaacaaagcgaagcgcccccgccgtatccgacccagcgcgtggattatggctggctttaccagacccgctggcccctgttgcggcgggctttcgcggggtttcgggcaagggcttcggcccaggataagacccgactggaagcctttatcgaggccgagcgcttctggctggaagactatgcgctctttatggccctcaagacccggtttgacggcaagccctggaacgagtggagccccgagctgcgcgaccgtgaaccggctgccctggccagggcccgtgaggagctggccgaggaggtggccctttacgagtggattcagtggcttttttatctggaatggggccagaccaaggcctatgccgaatccaaggggattcagattatcggcgatatgcccatctttgtggccttcgattcctcagatgtctgggccaacccgcagtacttctacctcgaggccgatggcaaccccacggtggtggcgggcgttccgccggactacttctccgaaaccggccagctctggggcaatccgctctatcgctgggatgtgatggaaagggacaactttgcctggtggattgcccgcataaggcagtcgctcaagcagtgccacctggtgcgcatcgaccacttccgcgggtttgaagcctactgggaggttccgtttggccggcccaatgctgtggaggggcgctgggtcaaagccccaggggagaagctgtttgctgcggtgcgggcccaactgagcgatgcgcccatcattgccgaagacctgggggtgatcacccccgaggtggaggctttgcgcgatggcttcgggttccccggcatgaagattttgcagtttgctttttccggtgaggacaacgcctttttgccccacaactaccccgcgcacggcaatgtggtggtgtacagcggaacccacgacaacgacaccaccctgggatggttccgcaccgcgccggaggccgagcgggccttcatgcgggcctacctggcccgctatggcatccgttgtttgtcggaatacgaggtcgcgggcgctttgatcgagctggccttcaaaagcccggccaagctggctattgtgcctttgcaggacgtgctggggctgggccccgaggcccgcatgaacttccccggacggctgggggacaactgggcgtggcgctacgccgaaggcgacctcgagcccggtctggccgcgggactgcgggccctggccgaggccagccagcgcgcttga

SEQ ID NO: 5 - protein, 692 aa, Aquifex aeolicus
MEEEKVKEGLWELAYNLWWTWNPPAKELFRSIDPLLWKETKENPIELLRKTKLLENKLKDEDFISHFKYVYSLYKTYMNRHSKYEDTYKKPIVFLSPEYGLHHTLLIYAGGLGFLAGDILKESSDLGFPLIGVGFMYPQGYVKQRIRVDGWQEDLDAQNQKELMPVKKVLDKEGKWLKCYVYVRDEKVYFGVWEVNVGKTKLYLLDTNVEENTPWNREISSRLYVPDKDLRLRQQIVLGFGTVILLEKLGIDAGGFHINEDYPSFVFLAEIFKLLKKGLTWDKAIEEVRKISLFTTHTPLRVAVNTYPFHMIEEQFLFVKDVYGIDVKKVLELGTNPEDPSEGFNSTIMSLRLAKYVNAVSKRHQEVSSKMWSFLFKEKENPIDYVTNGVHFPTWICSDLRRLYEEYLGENFVELHDHKSLWELIRDIPDEELWEYHIRNKERLIEHIKDRARERWVKEKADPSILMAEGLFLDSDVLTVGFARRMTGYKRPDLIFTDVERLKKIVNDSERPVQIIFAGKAHPADIEGKKIIQRIFNFAKDPEFGGRIAFVEDYDELLAHYMVRGVDVWLNNPLPPLEACGTSGMKASMNGVLHLSILDGWWIEGYNGKNGWAFGDYEVEGDRNRADAEAIYNILENEVIPLYYERDERGVPVKWISMMKEAIKSITPNFCSRRMLKDYINKFYSKILKEEG

SEQ ID NO: 6 - DNA, 2079 bp, Aquifex aeolicus
  source 1..2079: mol_type = other DNA
atggaagaagaaaaagtgaaagaaggcctgtgggaactggcgtataacctgtggtggacctggaacccgccggcgaaagaactgtttcgcagcattgatccgctgctgtggaaagaaaccaaagaaaacccgattgaactgctgcgcaaaaccaaactgctggaaaacaaactgaaagatgaagattttattagccattttaaatatgtgtatagcctgtataaaacctatatgaaccgccatagcaaatatgaagatacctataaaaaaccgattgtgtttctgagcccggaatatggcctgcatcataccctgctgatttatgcgggcggcctgggctttctggcgggcgatattctgaaagaaagcagcgatctgggctttccgctgattggcgtgggctttatgtatccgcagggctatgtgaaacagcgcattcgcgtggatggctggcaggaagatctggatgcgcagaaccagaaagaactgatgccggtgaaaaaagtgctggacaaagaaggtaaatggctgaaatgctatgtgtatgtgcgtgatgagaaagtgtattttggtgtgtgggaagtgaatgtgggcaaaacaaaactgtatctgctggataccaatgtggaagaaaataccccgtggaatcgtgaaattagcagccgtctgtatgttccggataaagatctgcgtctgcgtcagcagattgttttaggttttggcaccgttatcctgttagaaaaactgggcattgatgcaggcggttttcatatcaatgaagattatccgagctttgtgtttctggccgaaatctttaaactgctgaagaaaggcctgacctgggataaagcaattgaagaagttcgtaaaatcagcctgtttaccacacatacaccgctgcgtgttgcagttaatacctatccgtttcacatgatcgaagaacagtttctgtttgtgaaagatgtgtatggcatcgacgtgaaaaaagttttagaactgggcaccaatccggaagatccgagcgaaggttttaatagcaccattatgagcctgcgtctggcgaaatatgttaatgcagttagcaaacgtcatcaagaggttagcagcaaaatgtggtcctttctgttcaaagaaaaagaaaaccccatcgactatgtgaccaatggtgttcattttccgacctggatttgtagcgacctgcgtcgcctgtatgaagaatatctgggtgaaaattttgtggaactgcacgatcataaaagcctgtgggaactgattcgtgatattcctgatgaagaactgtgggaatatcatatccgtaataaagaacgcctgatcgagcatattaaagatcgtgcacgtgaacgttgggttaaagagaaagccgatccgagcattctgatggcagaaggtctgtttctggatagtgatgttctgaccgttggttttgcacgtcgtatgaccggttataaacgtccggatctgatttttaccgatgttgaacgtctgaaaaaaatcgtgaatgatagcgaacgtccggtgcagattatctttgcaggtaaagcacatccggcagatattgaaggcaaaaaaatcattcagcgcatctttaactttgcgaaagatccggaatttggtggtcgtattgcattcgtggaagattatgatgagctgctggcacattatatggttcgtggtgttgatgtgtggctgaataatccgctgcctccgctggaagcatgtggcaccagcggtatgaaagcaagcatgaatggtgtgctgcatctgagtattctggatggttggtggattgaaggttataatggtaaaaatggttgggcctttggcgattatgaagttgaaggtgatcgtaatcgtgcagatgcagaagccatttataacatcctggaaaacgaagtgatcccgctgtattatgaacgtgatgaacgcggtgttccggttaaatggattagcatgatgaaagaagccatcaaaagcatcaccccgaatttttgtagccgtcgtatgctgaaagattacatcaacaaattctatagcaaaatcctgaaagaagaaggttaa

SEQ ID NO: 7 - protein, 838 aa, Meiothermus ruber
MNVIGRIVSMPSLPEALKGLGELAYNLWWSWSPEAQHLFEQINPSQWKRFRANPVRALLEAEPERLTALAENAGYVGAVEATLARFHRYLQSRPQKPPRIAYFSMEYGFHESLPIYSGGLGILAGDHIKAASDLGLDLTAVGMFYHEGYFRQQLTPEGQQHEIYEDLRPEELPLVVVSKDGKPLKVGVEFPGRTVYVMAYKAQVGTIPVYLMSTNLPENRPEDRALTARLYAPGQEIRIEQEMILGIGGVRLLRALGLAPEVWHMNEGHAAFLGLERMREMVAAGSSFGEALEATSAGALFTTHTPVPAGHDSFPLDLVERYLDGWWNKLGISKEEFIALGREEKSYGPVFSMSNLALHTSRAAGGVSALHGEVSREMFKHLWKGLEPEEVPIGHITNGIHTFSFLHPEMHALYERSFPKTWAEQLHDPSQWTVERLEESELWHIRNKLRAHLVEEVRARLFEQRRRNGDLPASLRAAEKVLDPTVLTIGFARRFATYKRAILMFTDPDRLVSILNGPLPVQFVFAGKAHPKDEPGKEFIKKLAEKIKGLGLEDKMILLEDYDIGLARTLVQGVDVWLNTPRRPMEASGTSGMKAALNGALNFSVLDGWWAEAFNTTNGWAIGDGRTYATEEAQDYADAQSFYDTLQYKIIPLFYARGAVGTPSGWLAMVRDSIRTCGPTYSAQRMVDEYHRKFYTPLAQRSAHLLEKNAAALKEVADWKKQVQSAWDNVKVWVEAPSTTINQPLQLRAFVQAYGVPTKTLRVELVVRRNSGDLEVVALQHAGQENDALLYTGSYHPARPGSYEYGVRVVATHPELSSPREVTFVKWAGAVVEEPVKV

SEQ ID NO: 8 - DNA, 2517 bp, Meiothermus ruber
  source 1..2517: mol_type = genomic DNA
atgaacgtaattggccgaatcgtcagcatgcccagcctacccgaagccctcaagggcctcggcgagctggcctacaacctgtggtggagctggagccccgaagcccagcacctcttcgagcagattaatccttcgcagtggaagcgcttccgtgctaatccggtacgggccttgctggaagccgagcccgagcgcctgaccgccctggccgagaacgccggctacgtgggcgcggtcgaggccaccttggcccgcttccaccgctacctgcaaagccgcccccaaaagcccccacgaatcgcttatttctcgatggagtacggcttccacgagtcgctgcccatctactcgggcggcctgggcatcctggccggcgaccacatcaaggccgcctccgacctggggctcgacctgaccgctgtcgggatgttctaccacgagggctactttcgccagcagctcacccccgagggccagcagcacgagatctacgaagacctgcggcccgaagagctaccgctggtggtggtcagcaaggacggcaagcccctcaaggtgggggtggagtttcccggacgcaccgtatatgtgatggcttacaaggcgcaggtaggcaccattccggtctacctgatgagcaccaacctgcccgaaaaccggcccgaagaccgcgccctcaccgcaaggctctacgcccccgggcaggaaatccgcattgagcaggagatgattctgggtattggcggggtgcggctgttgcgggccctgggcctggcccccgaggtctggcacatgaacgagggccacgcggcctttttgggcctcgagcgcatgcgcgagatggtggctgccggaagctcctttggcgaggccctcgaggccacctcggcaggggcgctcttcaccacccacacccccgtacccgccggccacgacagcttcccgctggatctggtggagcgctacctggacggctggtggaacaagctgggcatcagcaaggaggagtttatcgccctgggccgcgaggaaaaaagctacggcccggtcttcagcatgtccaacctggccctccacacctcccgcgccgccgggggggtctcggccctgcacggcgaggtctcgcgcgagatgttcaagcacctgtggaagggcctcgagcccgaggaagttcccatcgggcacatcaccaacggcattcacacctttagcttcctgcaccccgagatgcacgccctctacgagcgcagcttccccaaaacctgggccgagcagctccacgaccccagccagtggacggtggaacggctcgaggagagcgagctttggcatattcggaacaagctgcgggcacacctggtcgaggaggtgcgggcccggctcttcgagcagcgccgccgcaacggcgacctcccggccagcctgcgggcggcagaaaaggtgctcgacccaaccgtgctgaccatcggttttgcccgccgctttgccacctacaagcgggccatcctgatgttcaccgaccccgatcggctggtctccattttgaatggccccctgccggtgcagtttgtgttcgccggtaaagcccaccccaaggacgagcccggcaaggagttcatcaagaagctggccgagaaaatcaagggactgggcctcgaggacaagatgattctgctcgaggattacgacataggcctggcccgcaccctggtgcagggggtggacgtctggctcaacaccccccgccgccccatggaggcctcgggcacctcgggcatgaaggcggccctgaacggcgctttgaacttctcggttctggacggctggtgggccgaggctttcaacaccaccaacggctgggccattggcgacggtcgcacctacgccaccgaagaagcccaggattacgccgacgcccagagcttctacgataccctgcagtacaagatcatcccgctgttctacgcccggggcgcggtgggcacccccagcggctggctggctatggtgcgcgacagcatccgcacctgtggccccacctactcggcccagcgcatggtggacgagtatcaccgcaagttctataccccgctggcccagcgctcggcgcaccttctggagaaaaacgccgcagcactcaaagaagtagcagactggaaaaaacaggtgcaaagcgcctgggacaacgtaaaagtctgggtggaggccccctccaccaccatcaaccagcccctgcaactgcgggcctttgtgcaggcctacggcgtccctaccaagaccctacgggtcgaactggtggtgcggcgcaacagcggcgatctggaagtggtggccctccagcacgccggccaggagaacgacgccctgctctacaccggcagctaccacccggcccgccccggcagctacgagtacggggtgcgggtggtggcgacgcacccggaactctcgagcccccgcgaggtcactttcgtaaagtgggccggagctgtagtggaagagccggtgaaggtatag

SEQ ID NO: 9 - protein, 547 aa, Meiothermus ruber
MSLHPLAGQPAPHSLLVNLPRLVSSYYALKPDPLNPAQQVAFGTSGHRGTSLAGTFNEAHILAIAQAVAEYRAEHGITGPLFMGMDTHALSEAAWITAVEVLAANGVEVRVEEGRGYTPTPLVSHAILEYNRNRSSGLADGIVITPSHNPPQDGGFKYNPPNGGPADTGVTRVIQERANQILRDGLTEVRRWPLSRALEAVRAFDFVTPYVRQLESIVDMAAIKAAGVRIGVDPLGGSSLRVWQRIAEHYSLSLTVVNERIDPSFAFMTLDKDGKIRMDCSSPYAMASLIGLKDRFDVAIGNDPDADRHGIVTPDGLMNPNHYLAVCIHYLYQNRPGWPAGMGVGKTLVSSSMIDRVVHSLGRRLVEVPVGFKYFVQGLLSGTIGFGGEESAGASFVRMDGSAWSTDKDGIILGLLAAEILAKTGRSPSQHYRDLEARFGASVYTRIDAEANSAQKKVLANLSPELVTATELAGEPIQAKLTRAPGNNEPIGGLKVVTENAWFAARPSGTEDVYKIYAESFRGEAHLERVVQEARHLVGEAFRRAGV

SEQ ID NO: 10 - DNA, 1644 bp, Meiothermus ruber
  source 1..1644: mol_type = other DNA
atgagtctccatccgttagcgggccagcctgcaccacatagtctgttagtaaatttaccacgcctggtttcgtcctattacgcgctcaaaccggacccgttaaatcccgctcaacaagttgcattcggaacgtcggggcatcgtgggactagtctcgcaggaacgtttaatgaagcacatattcttgcaattgctcaagccgtcgccgaatatcgcgctgaacatggaatcactggccccctgttcatgggtatggacacgcatgccttgagcgaagccgcatggatcacagccgtagaagttctcgctgcgaacggcgtagaagtccgtgtagaagagggtcgtggttatactcccacaccattggttagtcatgcaattctggaatataatcgtaaccgttcgtcaggcttagcggatggtattgtaattacgccgtcacataatccgccgcaagatggtgggtttaagtataatccaccaaatggtgggccggcggacactggtgtcacgcgtgtcattcaagagcgcgcaaatcaaattctccgtgatggtttgacggaagtgcgtcgttggccgctgtctcgtgcgctcgaagccgtgcgcgcgtttgactttgttactccgtacgtccgtcagcttgagtctatcgttgatatggcggcgattaaagcggcaggggtgcgtatcggagtggaccctttaggtgggtcatctctccgcgtgtggcaacgtattgcggaacattattcgttgtcgttaacagtcgtgaatgagcgtatcgatccttctttcgcgtttatgacgcttgacaaggatggtaagatccgtatggattgttcctctccgtatgcaatggcatcgctgatcgggcttaaagatcgctttgatgttgcgattggtaatgatccggatgcggatcgtcatggtattgttacgcctgatggtttgatgaatccgaatcattatttagccgtctgtattcactatttataccagaatcgtccggggtggcctgcagggatgggcgtaggcaaaacattggttagttcgtctatgatcgatcgcgttgtacattcattgggtcgtcgtctcgtcgaagttcctgttggtttcaaatacttcgtacaaggcctgctgtccggcactattggtttcggcggtgaagaatcggccggcgcgtctttcgtacgtatggatggttctgcttggtccactgataaggatggaattattctcggccttcttgcggcggaaatccttgctaaaactggtcgtagcccgtctcaacattatcgtgatcttgaagcgcgtttcggtgcgtctgtttatacgcgtatcgacgcggaagcaaattctgctcaaaagaaagttcttgcaaatctgtcgccggaacttgtcacagcaactgaattagcgggcgaacctattcaagcaaaattaacgcgtgctccggggaataacgaaccgattggtggcctgaaagttgttacggaaaatgcatggtttgcagcgcgtcctagcggtacggaagatgtatataaaatctacgctgaatcatttcgcggtgaagcccatctggaacgtgttgttcaagaagcacgccatcttgtgggtgaagcgttccgtcgcgcaggcgtataa

SEQ ID NO: 11 - protein, 445 aa, Meiothermus ruber
MLRLDLANVLSERIGPKGIDWPSALAAHAQRLEAARDALWQRKSDPAEFLGWIDVPEDTETLRRVLRFREAQAWVEDLVVLGIGGSALGAQAVAAALGKGPVRLHFVDNVEPEPILELLRKLEPHKTLVNVISKSGSTAETMAAFLAFRRWLEDRLGPDWKRHVVVTTDPAKGVLRPYAQAEGLPAFEVPRAVGGRFSVTCPVGTLPLAFAEVDLENLLAGARKANEQARAALEHNLPAQTALLHHLFSQKGQNIVVFMPYSTRLRYLPDWFVQLHDESLGKMRDRAGQEVRTGTTAVRAIGTTDQHAQVQLFREGPHDKLINFVRLLNPSEDLEIPAVRGLEALDYLFGKSFFKLLDAEAKATAHALAKAGQPNYTLTLEQLDAYHLGWLLQHLMWQTAFLGELWNINAFDQPGVELGKEYTYALMGRRGWESLAQELRAEGVE

SEQ ID NO: 12 - DNA, 1338 bp, Meiothermus ruber
  source 1..1338: mol_type = other DNA
atgttacgcctggatctcgccaatgtcctgtcggaacgcatcggcccgaaaggtattgattggcccagcgcattagcagcccacgcacaacgtttagaggcagctcgtgacgccctttggcaacgcaaatctgacccggcagaatttcttggctggatcgatgtccctgaagatacggaaactctccgccgcgtcttgcgttttcgtgaagcacaagcatgggtagaagacctcgtagtattgggaatcggcggttcagctcttggagcgcaagccgtagcagcagcattaggcaagggacccgtccgtttgcacttcgtcgataacgttgagcccgagcctattttggaacttctccgcaaactggaaccgcacaagactcttgtgaatgtgattagtaaaagcggtagcacggcagaaacgatggccgcattccttgcatttcgtcgttggttggaagaccgtttgggccccgactggaaacgccacgttgttgtaactactgatccggcgaaaggggtgctccgtccatacgcgcaagcggaaggtctgccggcgtttgaagtcccacgtgccgttggcggtcgcttctcggttacgtgtcctgtagggactttgcccttagcattcgccgaagtggatttggagaatttattggctggcgcgcgtaaagctaatgagcaagcgcgtgcagcgctggaacataatctcccagctcaaacagcccttcttcatcatttattcagtcaaaagggtcaaaatattgttgtattcatgccgtattcgactcgtttacgttatcttcctgattggttcgttcagcttcatgatgaaagtttgggtaaaatgcgtgaccgcgcgggtcaagaggtccgtactgggacgactgcagtgcgcgcaattgggacgaccgatcaacatgcgcaagttcaactgtttcgtgaaggacctcatgataaactgattaacttcgttcgtttgctcaatccatcagaagacttggagatccctgcagtccgtggcttggaagcgctggattatctcttcgggaaatccttctttaaattgttggacgcggaagcgaaggcgacggcacatgctttagcgaaagcgggtcaaccgaattatactctgacgttagagcagctggacgcatatcatcttgggtggttactgcagcatctcatgtggcaaaccgcgttcttgggcgaattatggaatattaatgcgtttgatcaacctggcgttgagttgggtaaagaatatacgtatgcacttatgggccgtcgcggatgggaatcactcgcgcaagaacttcgtgccgagggtgttgagtga

SEQ ID NO: 13 - protein, 220 aa, Escherichia coli
MELYLDTSDVVAVKALSRIFPLAGVTTNPSIIAAGKKPLDVVLPQLHEAMGGQGRLFAQVMATTAEGMVNDALKLRSIIADIVVKVPVTAEGLAAIKMLKAEGIPTLGTAVYGAAQGLLSALAGAEYVAPYVNRIDAQGGSGIQTVTDLHQLLKMHAPQAKVLAASFKTPRQALDCLLAGCESITLPLDVAQQMISYPAVDAAVAKFEQDWQGAFGRTSI

SEQ ID NO: 14 - DNA, 663 bp, Escherichia coli
  source 1..663: mol_type = genomic DNA
atggaactgtatctggatacttcagacgttgttgcggtgaaggcgctgtcacgtatttttccgctggcgggtgtgaccactaacccaagcattatcgccgcgggtaaaaaaccgctggatgttgtgcttccgcaacttcatgaagcgatgggcggtcaggggcgtctgtttgcccaggtaatggctaccactgccgaagggatggttaatgacgcgcttaagctgcgttctattattgcggatatcgtggtgaaagttccggtgaccgccgaggggctggcagctattaagatgttaaaagcggaagggattccgacgctgggaaccgcggtatatggcgcagcacaagggctgctgtcggcgctggcaggtgcggaatatgttgcgccttacgttaatcgtattgatgctcagggcggtagcggcattcagactgtgaccgacttacaccagttattgaaaatgcatgcgccgcaggcgaaagtgctggcagcgagtttcaaaaccccgcgtcaggcgctggactgcttactggcaggatgtgaatcaattactctgccactggatgtggcacaacagatgattagctatccggcggttgatgccgctgtggcgaagtttgagcaggactggcagggagcgtttggcagaacgtcgatttaa

SEQ ID NO: 15 - protein, 235 aa, Methanocaldococcus jannaschii
MILLVSPIDVEEAKEAIAGGADIIDVKNPKEGSLGANFPWMIKAIREVTPKDLLVSATVGDVPYKPGTISLAAVGAAISGADYIKVGLYGVKNYYQAVELMKNVVRAVKDIDENKIVVAAGYADAYRVGAVEPLIVPKIARDAGCDVAMLDTAIKDGKTLFDFQSKEILAEFVDEAHSYGLKCALAGSIKKEHIPILKEIGTDIVGVRGAACKGGDRNNGRIDRELVKELKELCK

SEQ ID NO: 16 - DNA, 663 bp, Methanocaldococcus jannaschii; identical to SEQ ID NO: 14
  source 1..663: mol_type = other DNA

SEQ ID NO: 17 - protein, 236 aa, Methanococcus maripaludis
MILLVSPKDVAEAYEAIEGGADIIDVKNPPEGSLGANFPWVIKETRDATPEGMLVSAAIGDVPYKPGTVTLAALGATVSGADYIKIGLYGTRSYQEALDVMKNVTKAVKDAGENKIVVAAGYADAYRVGAVDPLVIPKVARDAGCDVAMLDTAVKDGKTLFDHMDLDLLREFVEETHKYGMKCALAGSIKIEEIPMLKEIGCDIVGVRGAACTKGDRNAGRIQKDLVKEIVKVCKD

SEQ ID NO: 18 - DNA, 711 bp, Methanococcus maripaludis
  source 1..711: mol_type = other DNA
atgattctgcttgtgtcaccgaaggacgtcgccgaggcttatgaagcgatcgagggcggggcggacatcattgacgttaagaacccgcctgagggtagccttggtgcgaactttccttgggtgattaaggaaacccgcgatgctaccccagaggggatgttagtgagcgctgccattggggacgtcccatataaaccaggcacggtaactctcgccgctctgggcgccacggtcagcggggcagactacattaaaatcggcctttacggcacccgtagctatcaagaggcgctcgatgttatgaagaacgtgaccaaggcggtaaaggacgccggcgaaaacaagattgtagttgccgccggatacgccgatgcctatcgtgtcggcgccgtggaccctttggttatccctaaggtggcacgcgacgccggttgcgatgttgcgatgcttgacacggccgttaaggacggcaagaccttattcgaccacatggatttagatctcttgcgtgaattcgtcgaggaaacccataagtacggaatgaagtgtgccctggccggtagcattaagatcgaggaaattcccatgttgaaggagattggttgtgacattgttggagtacgtggggccgcatgtacgaagggcgaccgtaatgctggccgtatccaaaaggatcttgtcaaagagattgtaaaggtatgcaaggactga

SEQ ID NO: 19 - protein, 235 aa, Methanothermococcus okinawensis
MILLVSPKDVNEAIETIKGGADIVDVKNPPEGSLGANFPWIIKEIREITPKNLFVSAAIGDVPYKPGTVALAALGAAMSGADYIKVGLYGTKSYNEAVDLMEKVVKAVKGVDENKIVVAAGYADAHRVGAVEPLIVPKIARDAGCDVAMLDTAVKDGKTLFDHLNEKILAEFVEETHSYGLKCALAGSIKKEEIPILKDINCDIVGVRGAACTKGDRNNGTIKSELVKELSKLCK

SEQ ID NO: 20 - DNA, 708 bp, Methanothermococcus okinawensis
  source 1..708: mol_type = other DNA
atgattttgctcgtatcaccaaaggatgtaaatgaagccatcgaaaccattaagggtggagcggatatcgtggatgtaaagaatccccctgaaggctcccttggagcgaatttcccgtggattatcaaggagatccgcgagatcacgccaaagaacctgttcgtctccgcggctatcggcgatgtgccgtataaaccaggtacagttgcccttgccgccttaggcgccgcaatgtcgggtgcggactacatcaaagttggtttgtatgggactaagagctacaatgaggcagtggacttgatggagaaggtcgtgaaggcggtcaagggagttgacgaaaataaaatcgttgtcgcggcgggctacgctgatgctcaccgcgtcggggccgtcgaaccccttattgttcctaagattgcacgcgacgccggttgcgatgtagcaatgctggatactgccgtaaaggacggtaagaccctgttcgaccatctgaatgagaagattctggccgagtttgtagaagagacacattcctacggtttaaaatgcgcacttgcggggagcattaagaaggaagagatccccattttaaaagatattaactgcgatattgtgggtgtccgcggtgcggcctgcacgaagggcgaccgtaacaatggcaccatcaagagcgagctggtaaaggagctgtcaaagttatgcaaatga

SEQ ID NO: 21 - protein, 237 aa, Methanobacterium paludis
MLLLISPINTEEALEAVEGSADIIDVKNPKEGSLGANFPWVIKSIRELTPEAMHVSATIGDVPYKPGTVSLAAAGAVVSGADYIKVGLYGTKNYDEALEVMKNVVKSVREFDHDALVVASGYADAHRVGAVDPMEIPRVAAESGADIAMVDTAVKDGKTLFDFMDKDALTKFTDDTHKYGLKVALAGSVKAEQLEMLYDIGCDIVGIRGAACVGGDRNTGKIHRSAVSKLKKMIENF

SEQ ID NO: 22 - DNA, 714 bp, Methanobacterium paludis
  source 1..714: mol_type = other DNA
atgttactcctcatttcccctatcaatactgaggaagccctggaagccgttgaggggtcggcagacatcatcgatgttaagaaccctaaggaaggcagcctgggtgcgaacttcccttgggttattaaatcgattcgtgagttaacacccgaggctatgcatgtgtccgcgacgatcggtgacgtcccttataagccggggacggtatcgctggccgccgctggtgcggttgtgtcaggcgcagattatattaaggtgggcctttatgggacgaagaattatgatgaggcgttagaggtgatgaagaatgtagtcaaatcagtgcgtgagtttgatcatgacgcgctggttgttgctagtggttacgccgacgcgcaccgtgtcggcgcagtcgaccctatggagatccctcgcgttgccgcagagtctggagcagacatcgcaatggtggacactgcggttaaggacggtaagacgctcttcgatttcatggacaaggacgccctgacgaagttcacggacgatactcataagtatgggctgaaggtcgcccttgcgggtagcgttaaggccgagcaattagagatgttatacgacatcgggtgcgacatcgtgggcattcgtggcgcagcctgcgtcggcggtgatcgcaatacgggtaaaatccatcgtagtgccgtcagtaagttaaagaagatgatcgaaaatttctga

SEQ ID NO: 23 - protein, 238 aa, Methanobrevibacter wolinii
MLLLISPINHEEAVEAIEGGADIVDVKNPKEGSLGANFPWVIKDIRSITPSDKLVSATIGDVPYKPGTVSLASLGALVSGADYIKVGLYGTQNYEQAVEVMKNVVKTVKDESPDTIVVAAGYADADRVGAVSPWDIPKVARDSGADLAMLDTAVKDGKTLFDFMTMEDLEKWVAEAQEYDLKTALAGSVKKEQLKPLNDLNCDVVGIRGAACVDGDRNTGHIDRTAVKGLKDLVDSFN

SEQ ID NO: 24 - DNA, 717 bp, Methanobrevibacter wolinii
  source 1..717: mol_type = other DNA
atgctgttgttaatcagcccaatcaaccacgaagaggccgttgaggctatcgaaggtggcgcagatattgttgacgtaaagaatcctaaggaaggttcacttggggcgaatttcccttgggtcattaaggatattcgctctatcacgccttcagacaagctggtttcggcgacgattggcgacgtaccgtacaaacccggtacggtgagtctggcgtcacttggcgcccttgtatctggggcggattatatcaaggttggtctttacggtacccaaaactacgaacaggccgtcgaggtcatgaagaatgtcgtaaagaccgtgaaggacgagtcccctgacacaatcgtcgtagcggcaggttacgcggacgcggatcgcgtcggtgcggtttccccctgggatattccaaaggtagcgcgtgatagcggcgcggacttggccatgcttgataccgctgtgaaggatggcaagactttattcgattttatgacgatggaagatctggagaaatgggtggcggaagcacaagaatatgatctgaaaaccgcgttagccggttccgtaaagaaggagcaactgaagccgctgaacgacttgaattgcgatgtcgtgggtatccgtggcgcggcctgtgtggatggagatcgcaacaccgggcacatcgaccgcactgcggttaaggggttgaaggatttagtggactcattcaattga

SEQ ID NO: 25 - protein, 246 aa, Methylomonas methanica
MSGMLASVNSLDEALLIQSFSVDIVDLKQPAQGALGALSVSEVAEIVANLSGRNVISATVGDLPMQPDLLFTAVQAMASTGVDYVKIGFFPGGDWQACIDSLATLARTYRLIAVLFADTGPDVGIINALRKAGFAGVMLDTMDKTLGSLTQLMTWSELAGFTDAAKAAGLLTGLAGSLTQHDIPALLSLQADYLGFRGALCRQHCRTAQLDADRIVWIRQLLLGAGQPNGAMGLQSRSAELNVLGG

SEQ ID NO: 26 - DNA, 741 bp, Methylomonas methanica
  source 1..741: mol_type = other DNA
atgtcaggcatgttagccagcgtgaattctttagacgaggcgttacttatccaatcattctccgtggacatcgtggatttgaagcaaccagcgcaaggggccctcggtgctctgtcggtatccgaggtggcagaaatcgtggcgaacctttcaggtcgcaacgtcattagcgctacagtaggggatttacctatgcaacctgacctgcttttcaccgcagttcaagcgatggcttcaacgggcgtggactatgtgaagattggattctttccgggcggcgattggcaggcatgtattgactcgttagcgacgctggcacgcacataccgcttaattgctgttctctttgccgatacggggcccgatgtgggaattatcaacgccttacgcaaggccgggtttgcgggtgtgatgctcgatacaatggataaaacgttggggtctttgacgcaattaatgacatggagcgagctggcgggcttcactgatgcggccaaggcagcgggcctgctgacggggcttgcgggtagcttaacccagcacgacattcctgcccttcttagcttgcaagccgattatctgggctttcgcggcgcgttgtgtcgccagcattgtcgtacggcgcagctcgacgcagatcgcattgtgtggattcgtcaattactgttgggtgccggtcaaccaaatggcgctatggggctgcagagccgtagcgcagagcttaacgtattaggcgggtaa

SEQ ID NO: 27 - protein, 234 aa, Methanosarcina mazei
MKLLVSPINSEEAIIASIGGADIVDVKNPKEGSLGANFPWVIREVKAVVNGRQPISATIGDFNYKPGTAALAALGAAVAGADYIKVGLYDIQTESQALELLTKITRAVKDYDPLKKVVASGYSDYKRINSISPLLLPAVAAEAGVDVVMVDTGVKDGKSTFEFMDEKELKEFTDLAHRYGLENAIAGSLKFEDIPLLERIGPDIIGVRGMVCGGDRSTSIRQELVEKLVAECQA

SEQ ID NO: 28 - DNA, 705 bp, Methanosarcina mazei
  source 1..705: mol_type = other DNA
atgaagttgttagtaagtcccatcaattccgaagaagctattattgcctctatcggcggcgcagacattgtggacgtgaagaacccaaaggaaggaagtctcggcgcgaacttcccttgggtaattcgcgaggtcaaggctgttgtcaacggtcgccaaccgatcagtgccaccatcggtgatttcaactacaagccgggtacggccgcgttggcagcattaggtgcggctgtcgccggggctgactacatcaaggtaggtctgtacgacatccaaacagagagccaagcgttggagcttctgacgaagatcacccgcgcggtgaaggactatgacccgttgaagaaggtagtggcgagtggttacagcgactataagcgtattaattctatttcaccgcttttattgccggccgtggctgctgaggccggggtggacgtggtgatggttgacacgggtgttaaggatggcaagtccacgttcgagttcatggatgagaaggagttgaaggaattcaccgatcttgcgcaccgttatggtttagagaatgcgattgcaggctcgctgaagtttgaggatatccccttgttagagcgcattggcccagacattatcggagttcgtggaatggtctgtggcggagatcgctctacatcgatccgtcaggagttagtggagaagttagttgccgagtgtcaagcctaa

SEQ ID NO: 29 - protein, 236 aa, Methanothermococcus thermolithotrophicus
MIILVSPKDVNEAIEAIEGGADIIDVKNPPEGSLGANFPWVIKQIKEVTPENRLVSATIGDVPYKPGTASLAALGACVSGADYIKVGLYGTKSYSQSLDLMEKVTKAVKDFDEKKIVVAAGYADAYRVGAVDPLVIPKIARDAGCDVAMLDTAVKDGKTLFDHLNEKLLEEFINETHAYGMKCALAGSIKKEEIPILKDIGCDIVGVRGAACTKGDRNEGRIQRNLVNELVKLCRD

SEQ ID NO: 30 - DNA, 711 bp, Methanothermococcus thermolithotrophicus
  source 1..711: mol_type = other DNA
atgatcattctcgttagcccgaaggacgtgaacgaagcgattgaggcgatcgagggcggtgcggacatcatcgatgttaagaatccgccagagggttctttaggagcaaattttccctgggttatcaaacaaatcaaagaagtaactccagagaaccgtttggtatcagctacgatcggagacgtcccctacaagccaggaactgcgtctttggcggcactgggagcctgtgtatcaggcgccgattatattaaagtaggtctttacggcactaagtcatactcgcaaagcctcgacctgatggaaaaggtcacgaaggcagtaaaggacttcgacgaaaagaagattgtagttgcggcgggttacgcggacgcgtatcgtgttggtgcggtggacccactcgttattccaaagatcgcgcgtgacgcgggttgcgacgttgctatgttagacaccgccgtaaaggatggcaagaccctgttcgatcatctgaatgagaaacttttggaagaattcatcaatgaaacacacgcctatggcatgaagtgtgctttggccggttcgatcaagaaagaggagattcctattttaaaagacatcggttgcgatattgttggggtgcgcggggccgcctgcacgaaaggtgaccgcaacgaaggtcgcattcaacgcaaccttgtcaacgaactcgttaagctgtgccgtgattaa

SEQ ID NO: 31 - protein, 271 aa, Escherichia coli
MSVKVIVTDMDGTFLNDAKTYNQPRFMAQYQELKKRGIKFVVASGNQYYQLISFFPELKDEISFVAENGALVYEHGKQLFHGELTRHESRIVIGELLKDKQLNFVACGLQSAYVSENAPEAFVALMAKHYHRLKPVKDYQEIDDVLFKFSLNLPDEQIPLVIDKLHVALDGIMKPVTSGFGFIDLIIPGLHKANGISRLLKRWDLSPQNVVAIGDSGNDAEMLKMARYSFAMGNAAENIKQIARYATDDNNHEGALNVIQAVLDNTSPFNS

SEQ ID NO: 32 - DNA, 816 bp, Escherichia coli
  source 1..816: mol_type = genomic DNA
atgagcgtaaaagttatcgtcacagacatggacggtacttttcttaacgacgccaaaacgtacaaccaaccacgttttatggcgcaatatcaggaactgaaaaagcgcggcattaagttcgttgttgccagcggtaatcagtattaccagcttatttcattctttcctgagctaaaggatgagatctcttttgtcgcggaaaacggcgcactggtttacgaacatggcaagcagttgttccacggcgaactgacccgacatgaatcgcggattgttattggcgagttgctaaaagataagcaactcaattttgtcgcctgcggtctgcaaagtgcatatgtcagcgaaaatgcccccgaagcatttgtcgcactgatggcaaaacactaccatcgcctgaaacctgtaaaagattatcaggagattgacgacgtactgttcaagttttcgctcaacctgccggatgaacaaatcccgttagtgatcgacaaactgcacgtagcgctcgatggcattatgaaacccgttaccagtggttttggctttatcgacctgattattcccggtctacataaagcaaacggtatttcgcggttactgaaacgctgggatctgtcaccgcaaaatgtggtagcgattggcgacagcggtaacgatgcggagatgctgaaaatggcgcgttattcctttgcgatgggcaatgctgcggaaaacattaaacaaatcgcccgttacgctaccgatgataataatcatgaaggcgcgctgaatgtgattcaggcggtgctggataacacatccccttttaacagctga

SEQ ID NO: 33 - protein, 261 aa, Eubacterium limosum
MVKLISADMDGTLLDSNKELSPELFPLIESLAEQGVRFAAASGRQYYNLEHIFEPVKDKMIFIAENGSVVFENDVNSFANVIDRETVQEIVKEIRKITGASPVICGLKGAYAESDEPELLENIKMYYRRYEIMDDILAVEDDICKIAVYDYVNAEINSHVPLLEAFGEQMEIAVSGEHWVDLSNPGCNKGTAISKIQEKYGISYEETMLFGDYLNDYEMMKTGKYSYAMENSHPQLKEICNYTAKSNDENGVVEAIRAYFK

SEQ ID NO: 34 - DNA, 786 bp, Eubacterium limosum
  source 1..786: mol_type = other DNA
atggtaaagttaatatctgccgacatggatggcacgctcctcgactccaacaaggagctgtctcccgagcttttcccgttaatcgagagcctggcagaacaaggggttcgttttgcagcagcctctggtcgacaatattacaacctggaacacatattcgagccagtcaaggataaaatgatcttcatagcggaaaacgggagtgttgttttcgagaacgatgtcaactctttcgcaaatgtgattgacagagaaaccgttcaagagatagtaaaagagatccgcaaaataactggggcgtcacctgtaatatgcggtttgaaaggtgcctacgctgaatcagatgaacctgagttattagagaacattaagatgtactatcgtcgttacgagattatggatgacatcctggctgtggaagatgacatttgtaagattgccgtgtacgactacgtgaacgccgagattaatagtcatgtaccgctccttgaggcgttcggcgaacaaatggaaattgctgtatcaggcgagcactgggtcgacctgtcgaacccgggatgcaacaagggcacagccatctcaaagattcaggagaagtacggcataagttacgaggagacgatgctgttcggcgattaccttaacgattacgagatgatgaagacaggcaagtacagttacgcaatggaaaattcgcaccctcagcttaaagaaatctgcaactacacagctaaatccaatgacgagaatggagtagtagaagcaattcgcgcctactttaagtaa

SEQ ID NO: 35 - protein, 266 aa, Blautia obeum
MIKLIVTDIDGTLVKDGTLDINPEYMDVIKKLTEKGIHFVACSGRQYCSERQLFAPVKDRIFFISDGGTLIRTSEKILKVHTLSAEIWKNMARMAKKEMPGCDYFISSPDVSYAENSKTPMFRWLHDSYGYDIREVPDLLKPSFENERIMKIAIYNTDHCEEKCAPVFTPYWKDKVNMACAGKEWMDCTPHGADKKSAVAFLQEYLGISPEETCTFGDNINDIEMLKNAGYSYAVANAREEVQAAAKAVCPSYLEDGVLSVLKTLL

SEQ ID NO: 36 - DNA, 801 bp, Blautia obeum
  source 1..801: mol_type = other DNA
atgattaaattgattgtaacggacatagatggtaccttggttaaagacggcacattagacatcaatcctgaatatatggatgtgattaagaagctgacggagaaaggtatacattttgtcgcttgctcgggcagacaatattgtagcgaacggcaactgttcgcgccggtgaaggatagaattttcttcatatcagacggtggtacattaattcggacgagcgaaaagattttaaaagtccacacactcagcgctgagatttggaagaacatggctagaatggccaagaaggagatgcccggatgcgactactttataagctccccggacgtgagttacgcggaaaacagtaagacaccgatgttccgctggctgcatgatagctacggttatgatattcgggaagtgccggatcttctgaagcccagcttcgagaacgagcgtattatgaaaatagcaatctacaatacagaccattgcgaggaaaagtgtgcaccagtattcactccctactggaaggataaggtcaacatggcgtgtgcaggaaaggaatggatggactgcacgccacacggtgcggacaagaagagcgcagttgcattcttacaagagtacttgggaatcagccctgaagaaacttgcaccttcggagataacattaacgacatcgagatgttgaagaatgccgggtatagttacgctgtcgcaaacgcaagagaagaggttcaagcggctgctaaagccgtgtgcccaagttatttagaggatggtgttctgtcagttcttaagacgttgctgtga

SEQ ID NO: 37 - protein, 281 aa, Weissella cibaria
MTIKLIATDMDGTLLRDDRTFDYARMEDLLDQLDEKGIRFVAASGNQYKQLRSYFEPVNPDRITYVSDNGALITHNNEVLAESSLSRDQIARVMQWNSETHANMDNLIILSGNDGAYVSNHATPEMIAAVKTFYPTVHQVEKFMDVDDNIFRFSLVWDPSVDVHEHVQQLREVFGEELHTTGSGFGSVDILAPGVNKRTGLEQLAAKWDIKPEEMAAFGDNGNDLEMLRYVKYPFVMPNAEDFMKVRVQNLAVNDNNHNGVLDTIEALLAGAYDDESVFDK

SEQ ID NO: 38 - DNA, 846 bp, Weissella cibaria
  source 1..846: mol_type = other DNA
atgaccattaaattgatagctacagacatggacggcacgcttctccgtgacgatcgtacgttcgattacgcacggatggaagatctgctggaccaactcgatgaaaagggtatacgttttgtcgccgcaagcggtaaccaatataagcagctgagatcctactttgagcctgtcaacccggatcggatcacgtacgtatcggataacggagcgcttattacccacaacaacgaggtactggcggagagtagcttgagtcgcgaccagatcgcacgcgttatgcagtggaactctgagacacacgccaatatggacaacctgattatcctgtctggaaacgacggtgcgtacgtttccaaccacgctacgcctgagatgatcgccgccgtaaagacattctacccgacggtccaccaggtggaaaagttcatggacgttgacgacaacatattccgattttctctggtatgggaccctagtgtagacgttcatgagcatgtacaacaactgcgggaagtatttggcgaggagttgcacacaaccggttctggtttcggctcggtcgatatactcgcgccaggcgttaacaagcggactggactggagcaattggccgctaaatgggacatcaaacccgaggagatggctgcattcggagataatggtaacgacctggagatgttacgttatgtcaagtacccttttgtaatgcccaacgcagaagacttcatgaaagtcagagtccaaaacttggcggtcaacgacaataaccataacggagtgttggacaccattgaggcccttttggcgggagcttacgacgatgagagtgtctttgataagtag

SEQ ID NO: 39 - protein, 336 aa, Clostridium thermocellum
MAVKIGINGFGRIGRLVFRASLNNPNVEVVGINDPFIDLEYMQYMLKYDTVHGQFKGEISQDNGKLVVNGRKISVYGFTDPAEIPWSECGAEYIVESTGVFTTTEKASAHFKGGAKKVVISAPSADAPMFVMGVNHDKYTKDMNVVSNASCTTNCLAPLAKVIHENFGIVEGLMTTVHATTATQKTVDGPSKKDWRGGRAAAGNIIPSSTGAAKAVGKVIPELNGKLTGMAFRVPTLDVSVVDLTCRLEKPATYDEIKAAVKKASENELKGILGYTEDAVVSSDFIGDPRTSIFDAEAGISLNSNFVKLVAWYDNEWGYSNKVVDLIVHMASVDAK

SEQ ID NO: 40 - DNA, 1011 bp, Clostridium thermocellum
  source 1..1011: mol_type = genomic DNA
atggcagtaaaaattggtatcaacggttttggacgtatcggtcgtcttgtgttcagggccagtctcaacaacccgaacgttgaggttgtaggtataaacgacccatttattgaccttgaatacatgcaatatatgttaaagtatgatacagtacatggtcagttcaaaggtgaaatttcacaagacaacggaaaactcgttgtaaacggcagaaaaataagtgtttatggtttcactgatcctgctgagattccgtggagcgaatgcggtgcggaatacatcgttgaatcaacgggtgtattcacaactactgaaaaggcttcagctcacttcaagggcggtgcaaagaaggtagttatcagtgctccttcggcagatgctccgatgtttgttatgggtgtaaaccatgataaatacacaaaggatatgaacgttgtatctaacgcttcatgtacaacaaactgccttgctcctctggctaaagttatacatgaaaacttcggaatcgtagaaggcttgatgactactgtacacgctacaactgcaactcaaaagactgttgacggtccttcaaagaaagactggagaggcggacgtgcagcagcaggcaacatcattccttcatcaacaggagctgcaaaggcagttggaaaggttatccctgaattgaacggtaagttgacaggtatggctttcagagttccgactcttgacgtatctgttgttgacttgacttgccgtcttgaaaaaccggctacttatgatgaaatcaaagccgctgttaagaaagcttcagaaaatgaacttaagggtattttgggatacactgaggatgcggttgtttcttcagacttcatcggcgatccccgcacttcaattttcgatgctgaagcaggtatttctctcaacagcaactttgtaaaacttgttgcctggtacgacaatgaatggggttattcaaacaaagttgttgatttgatagttcatatggcttcggttgatgcaaaataa

SEQ ID NO: 41 - protein, 220 aa, Escherichia coli; identical to SEQ ID NO: 13

SEQ ID NO: 42 - DNA, 663 bp, Escherichia coli; identical to SEQ ID NO: 14
  source 1..663: mol_type = genomic DNA

SEQ ID NO: 43 - protein, 258 aa, Escherichia coli
MPRFAANLSMMFTEVPFIERFAAARKAGFDAVEFLFPYNYSTLQIQKQLEQNHLTLALFNTAPGDINAGEWGLSALPGREHEAHADIDLALEYALALNCEQVHVMAGVVPAGEDAERYRAVFIDNIRYAADRFAPHGKRILVEALSPGVKPHYLFSSQYQALAIVEEVARDNVFIQLDTFHAQKVDGNLTHLIRDYAGKYAHVQIAGLPDRHEPDDGEINYPWLFRLFDEVGYQGWIGCEYKPRGLTEEGLGWFDAWR

SEQ ID NO: 44 - DNA, 777 bp, Escherichia coli
  source 1..777: mol_type = genomic DNA
atgcctcgttttgcagctaatttatccatgatgttcaccgaagtgccttttattgaacgcttcgccgcagcgcgaaaagccgggttcgatgctgtggaatttctgtttccctataactactccaccctgcaaatccaaaagcaactggagcaaaaccatctgacactggcgctgttcaataccgctcccggagatattaatgcgggggaatggggattatccgcccttcccggacgtgagcacgaagcacacgcagacatcgacctggcactggaatatgcattggcgctcaattgtgaacaagtccatgtgatggcaggcgtcgtgcccgctggcgaagatgctgaacggtaccgggcagtatttatcgataatatccgctacgctgccgaccgctttgcgccacacggcaagcgaatattagttgaagcactcagccccggcgttaagcctcattatctcttctccagccagtatcaggcactggctattgttgaagaggttgcgcgagataacgtgtttattcaactagatacttttcatgcgcaaaaagtagatggcaacctgacgcatttaatccgcgactacgccgggaaatatgcgcacgtacaaattgccggactacctgatcgacatgaaccggacgatggagaaatcaactatccgtggctgttccgcctgttcgatgaggtgggatatcagggctggatcggttgtgaatataaacctcgtggcctcaccgaagaagggcttggctggtttgacgcctggcgctaa

SEQ ID NO: 45 - protein, 259 aa, Polynucleobacter wuianus
MPKFAANLTMLFNEVPFLDRFEKASSAGFKAVEFLFPYPFAANEIKQKLDQNQLSLVLHNLPAGDWDAGERGIACLPDRKEEFRAGVAKAIEYAKVLGVHQLNCLAGKVPTGADQKLAHATFVENLRYAAAELKKNHLRLLIEPINTFDIPGFFLNITQQAIDILSEVGADNVFVQYDIYHAQRMEGELANTIEKHFEKIAHIQLADNPGRNEPGTGEINYAYLFNHLDRIGYKGWIGCEYKPATTTEAGLGWIKQFNS

SEQ ID NO: 46 - DNA, 780 bp, Polynucleobacter wuianus
  source 1..780: mol_type = other DNA
atgccaaagtttgccgcgaacctgacaatgttgttcaatgaggtaccatttctcgaccgctttgagaaggctagctctgctggtttcaaggctgtagagttccttttcccgtatccgttcgctgccaatgagatcaaacaaaagttggaccagaaccaattatccttggttcttcacaatctcccagcgggcgactgggacgcgggtgaacgaggaatcgcttgtctcccagatcgcaaagaggagttccgggcgggtgtcgctaaagccatagagtacgctaaggtactgggtgtgcatcaattaaactgcttagcgggaaaagtaccaactggcgcagaccaaaagttggctcatgctacgttcgtcgaaaacttacgttacgctgccgccgagttaaagaagaaccacttgagattactcattgagcctattaatacattcgacatcccggggttcttccttaatataacccaacaagccattgacatactgagcgaagtgggtgctgataacgtcttcgtccaatacgatatctaccacgcacaaagaatggaaggggaattagccaacactattgaaaagcacttcgaaaagatagcccacatacaactggctgacaaccctggtcgtaatgaacctgggacgggtgaaattaactacgcatatctcttcaatcacctcgatagaataggttataagggatggataggatgcgaatataagccggccactacgaccgaggctggtttaggttggataaaacagttcaactcatga

SEQ ID NO: 47 - protein, 271 aa, Escherichia coli
MSVKVIVTDMDGTFLNDAKTYNQPRFMAQYQELKKRGIKFVVASGNQYYQLISFFPELKDEISFVAEDGALVYEHGKQLFHGELTRHESRIVIGELLKDKQLNFVACGLQSAYVSENAPEAFVALMAKHYHRLKPVKDYQEIDDVLFKFSLNLPDEQIPLVIDKLHVALDGIMKPVTSGFGFIDLIIPGLHKANGISRLLKRWDLSPQNVVAIGDSGNDAEMLKMARYSFAMGNAAENIKQIARYATDDNNHEGALNVIQAVLDNTSPFNS

SEQ ID NO: 48 - DNA, 816 bp, Escherichia coli
  source 1..816: mol_type = genomic DNA
atgagcgtaaaagttatcgtcacagacatggacggtacttttcttaacgacgccaaaacgtacaaccaaccacgttttatggcgcaatatcaggaactgaaaaagcgcggcattaagttcgttgttgccagcggtaatcagtattaccagcttatttcattctttcctgagctaaaggatgagatctcttttgtcgcggaagatggcgcactggtttacgaacatggcaagcagttgttccacggcgaactgacccgacatgaatcgcggattgttattggcgagttgctaaaagataagcaactcaattttgtcgcctgcggtctgcaaagtgcatatgtcagcgaaaatgcccccgaagcatttgtcgcactgatggcaaaacactaccatcgcctgaaacctgtaaaagattatcaggagattgacgacgtactgttcaagttttcgctcaacctgccggatgaacaaatcccgttagtgatcgacaaactgcacgtagcgctcgatggcattatgaaacccgttaccagtggttttggctttatcgacctgattattcccggtctacataaagcaaacggtatttcgcggttactgaaacgctgggatctgtcaccgcaaaatgtggtagcgattggcgacagcggtaacgatgcggagatgctgaaaatggcgcgttattcctttgcgatgggcaatgctgcggaaaacattaaacaaatcgcccgttacgctaccgatgataataatcatgaaggcgcgctgaatgtgattcaggcggtgctggataacacatccccttttaacagctga

SEQ ID NO: 49 - protein, 271 aa, Escherichia coli
MSVKVIVTDMDGTFLNDAKTYNQPRFMAQYQELKKRGIKFVVASGNQYYQLISFFPELKDEISFVAEEGALVYEHGKQLFHGELTRHESRIVIGELLKDKQLNFVACGLQSAYVSENAPEAFVALMAKHYHRLKPVKDYQEIDDVLFKFSLNLPDEQIPLVIDKLHVALDGIMKPVTSGFGFIDLIIPGLHKANGISRLLKRWDLSPQNVVAIGDSGNDAEMLKMARYSFAMGNAAENIKQIARYATDDNNHEGALNVIQAVLDNTSPFNS

SEQ ID NO: 50 - DNA, 816 bp, Escherichia coli
  source 1..816: mol_type = genomic DNA
atgagcgtaaaagttatcgtcacagacatggacggtacttttcttaacgacgccaaaacgtacaaccaaccacgttttatggcgcaatatcaggaactgaaaaagcgcggcattaagttcgttgttgccagcggtaatcagtattaccagcttatttcattctttcctgagctaaaggatgagatctcttttgtcgcggaagagggcgcactggtttacgaacatggcaagcagttgttccacggcgaactgacccgacatgaatcgcggattgttattggcgagttgctaaaagataagcaactcaattttgtcgcctgcggtctgcaaagtgcatatgtcagcgaaaatgcccccgaagcatttgtcgcactgatggcaaaacactaccatcgcctgaaacctgtaaaagattatcaggagattgacgacgtactgttcaagttttcgctcaacctgccggatgaacaaatcccgttagtgatcgacaaactgcacgtagcgctcgatggcattatgaaacccgttaccagtggttttggctttatcgacctgattattcccggtctacataaagcaaacggtatttcgcggttactgaaacgctgggatctgtcaccgcaaaatgtggtagcgattggcgacagcggtaacgatgcggagatgctgaaaatggcgcgttattcctttgcgatgggcaatgctgcggaaaacattaaacaaatcgcccgttacgctaccgatgataataatcatgaaggcgcgctgaatgtgattcaggcggtgctggataacacatccccttttaacagctga

SEQ ID NO: 51 - protein, 271 aa, Escherichia coli
MSVKVIVTDMDGTFLNDAKTYNQPRFMAQYQELKKRGIKFVVASGNQYYQLISFFPELKDEISFVAENGALVYEHGKQLFHGELTRHESRIVIGELLKDKQLNFVACGLQSAYVSENAPEAFVALMAKHYHRLKPVKDYQEIDDVLFKFSLNLPDEQIPLVIDKLHVALDGIMKPVTNGFGFIDLIIPGLHKANGISRLLKRWDLSPQNVVAIGDSGNDAEMLKMARYSFAMGNAAENIKQIARYATDDNNHEGALNVIQAVLDNTSPFNS

SEQ ID NO: 52 - DNA, 816 bp, Escherichia coli
  source 1..816: mol_type = genomic DNA
atgagcgtaaaagttatcgtcacagacatggacggtacttttcttaacgacgccaaaacgtacaaccaaccacgttttatggcgcaatatcaggaactgaaaaagcgcggcattaagttcgttgttgccagcggtaatcagtattaccagcttatttcattctttcctgagctaaaggatgagatctcttttgtcgcggaaaacggcgcactggtttacgaacatggcaagcagttgttccacggcgaactgacccgacatgaatcgcggattgttattggcgagttgctaaaagataagcaactcaattttgtcgcctgcggtctgcaaagtgcatatgtcagcgaaaatgcccccgaagcatttgtcgcactgatggcaaaacactaccatcgcctgaaacctgtaaaagattatcaggagattgacgacgtactgttcaagttttcgctcaacctgccggatgaacaaatcccgttagtgatcgacaaactgcacgtagcgctcgatggcattatgaaacccgttaccaatggttttggctttatcgacctgattattcccggtctacataaagcaaacggtatttcgcggttactgaaacgctgggatctgtcaccgcaaaatgtggtagcgattggcgacagcggtaacgatgcggagatgctgaaaatggcgcgttattcctttgcgatgggcaatgctgcggaaaacattaaacaaatcgcccgttacgctaccgatgataataatcatgaaggcgcgctgaatgtgattcaggcggtgctggataacacatccccttttaacagctga

SEQ ID NO: 53 - protein, 271 aa, Escherichia coli
MSVKVIVTDMDGTFLNDAKTYNQPRFMAQYQELKKRGIKFVVASGNQYYQLISFFPELKDEISFVAENGALVYEHGKQLFHGELTRHESRIVIGELLKDKQLNFVACGLQSAYVSENAPEAFVALMAKHYHRLKPVKDYQEIDDVLFKFSLNLPDEQIPLVIDKLHVALDGIMKPVTMGFGFIDLIIPGLHKANGISRLLKRWDLSPQNVVAIGDSGNDAEMLKMARYSFAMGNAAENIKQIARYATDDNNHEGALNVIQAVLDNTSPFNS

SEQ ID NO: 54 - DNA, 816 bp, Escherichia coli
  source 1..816: mol_type = genomic DNA
atgagcgtaaaagttatcgtcacagacatggacggtacttttcttaacgacgccaaaacgtacaaccaaccacgttttatggcgcaatatcaggaactgaaaaagcgcggcattaagttcgttgttgccagcggtaatcagtattaccagcttatttcattctttcctgagctaaaggatgagatctcttttgtcgcggaaaacggcgcactggtttacgaacatggcaagcagttgttccacggcgaactgacccgacatgaatcgcggattgttattggcgagttgctaaaagataagcaactcaattttgtcgcctgcggtctgcaaagtgcatatgtcagcgaaaatgcccccgaagcatttgtcgcactgatggcaaaacactaccatcgcctgaaacctgtaaaagattatcaggagattgacgacgtactgttcaagttttcgctcaacctgccggatgaacaaatcccgttagtgatcgacaaactgcacgtagcgctcgatggcattatgaaacccgttaccatgggttttggctttatcgacctgattattcccggtctacataaagcaaacggtatttcgcggttactgaaacgctgggatctgtcaccgcaaaatgtggtagcgattggcgacagcggtaacgatgcggagatgctgaaaatggcgcgttattcctttgcgatgggcaatgctgcggaaaacattaaacaaatcgcccgttacgctaccgatgataataatcatgaaggcgcgctgaatgtgattcaggcggtgctggataacacatccccttttaacagctga

SEQ ID NO: 55 - protein, 270 aa, Escherichia coli
MAIKLIAIDMDGTLLLPDHTISPAVKNAIAAARARGVNVVLTTGRPYAGVHNYLKELHMEQPGDYCITYNGALVQKAADGSTVAQTALSYDDYRFLEKLSREVGSHFHALDRTTLYTANRDISYYTVHESFVATIPLVFCEAEKMDPNTQFLKVMMIDEPAILDQAIARIPQEVKEKYTVLKSAPYFLEILDKRVNKGTGVKSLADVLGIKPEEIMAIGDQENDIAMIEYAGVGVAMDNAIPSVKEVANFVTKSNLEDGVAFAIEKYVLN

SEQ ID NO: 56 - DNA, 813 bp, Escherichia coli
  source 1..813: mol_type = genomic DNA
atggctattaaactcattgctatcgatatggatggcacccttctgctgcccgatcacaccatttcacccgccgttaaaaatgcgattgccgcagctcgcgcccgtggcgtgaatgtcgtgctaacgacgggtcgcccgtatgcaggtgtgcacaactacctgaaagagctgcatatggaacagccgggcgactactgcattacttataacggcgcgctggtacagaaggccgctgatggtagcaccgtggcgcaaactgctctcagctatgacgactatcgtttcctggaaaaactctctcgcgaagtcggttctcatttccacgccctggaccgcaccacgctgtacaccgccaaccgtgatatcagctactacacggtgcatgaatccttcgttgccaccattccgctggtgttctgcgaagcggagaaaatggaccccaatacccagttcctgaaagtgatgatgattgatgaacccgccatcctcgaccaggctatcgcgcgtattccgcaggaagtgaaagagaaatataccgtgctgaaaagtgcgccgtacttcctcgaaatcctcgataaacgcgttaacaaaggtacgggggtgaaatcactggccgacgtgttaggtattaaaccggaagaaatcatggcgattggcgatcaggaaaacgatatcgcaatgattgaatatgcaggcgtcggtgtggcgatggataacgctattccttcagtgaaagaagtggcgaactttgtcaccaaatctaaccttgaagatggcgtggcgtttgctattgagaagtatgtgctgaattaa

SEQ ID NO: 57 - protein, 199 aa, Escherichia coli
MLYIFDLGNVIVDIDFNRVLGAWSDLTRIPLASLKKSFHMGEAFHQHERGEISDEAFAEALCHEMALPLSYEQFSHGWQAVFVALRPEVIAIMHKLREQGHRVVVLSNTNRLHTTFWPEEYPEIRDAADHIYLSQDLGMRKPEARIYQHVLQAEGFSPSDTVFFDDNADNIEGANQLGITSILVKDKTTIPDYFAKVLC

SEQ ID NO: 58 - DNA, 600 bp, Escherichia coli
  source 1..600: mol_type = genomic DNA
atgctctatatctttgatttaggtaatgtgattgtcgatatcgactttaaccgtgtgctgggagcctggagcgatttaacgcgtattccgctggcatcgcttaagaagagttttcatatgggggaggcgtttcatcagcatgagcgtggggaaattagcgacgaagcgttcgcagaggcgctgtgtcatgagatggctctaccgctaagctacgagcagttctctcacggctggcaggcggtgtttgttgcgctgcgcccggaagtgatcgccatcatgcataaactgcgtgagcaggggcatcgcgtggtggtgctttccaataccaaccgcctgcataccaccttctggccggaagaatacccggaaattcgtgatgctgctgaccatatctatctgtcgcaagatctggggatgcgcaaacctgaagcacgaatttaccagcatgttttgcaggcggaaggtttttcacccagcgatacggtctttttcgacgataacgccgataatatagaaggagccaatcagctgggcattaccagtattctggtgaaagataaaaccaccatcccggactatttcgcgaaggtgttatgctaa

SEQ ID NO: 59 - protein, 432 aa, Escherichia coli
MKAILIPFLSLLIPLTPQSAFAQSEPELKLESVVIVSRHGVRAPTKATQLMQDVTPDAWPTWPVKLGWLTPRGGELIAYLGHYQRQRLVADGLLAKKGCPQSGQVAIIADVDERTRKTGEAFAAGLAPDCAITVHTQADTSSPDPLFNPLKTGVCQLDNANVTDAILSRAGGSIADFTGHRQTAFRELERVLNFPQSNLCLKREKQDESCSLTQALPSELKVSADNVSLTGAVSLASMLTEIFLLQQAQGMPEPGWGRITDSHQWNTLLSLHNAQFYLLQRTPEVARSRATPLLDLIKTALTPHPPQKQAYGVTLPTSVLFIAGHDTNLANLGGALELNWTLPGQPDNTPPGGELVFERWRRLSDNSQWIQVSLVFQTLQQMRDKTPLSLNTPPGEVKLTLAGCEERNAQGMCSLAGFTQIVNEARIPACSL

SEQ ID NO: 60 - DNA, 1299 bp, Escherichia coli
  source 1..1299: mol_type = genomic DNA
atgaaagcgatcttaatcccatttttatctcttctgattccgttaaccccgcaatctgcattcgctcagagtgagccggagctgaagctggaaagtgtggtgattgtcagtcgtcatggtgtgcgtgctccaaccaaggccacgcaactgatgcaggatgtcaccccagacgcatggccaacctggccggtaaaactgggttggctgacaccgcgcggtggtgagctaatcgcctatctcggacattaccaacgccagcgtctggtagccgacggattgctggcgaaaaagggctgcccgcagtctggtcaggtcgcgattattgctgatgtcgacgagcgtacccgtaaaacaggcgaagccttcgccgccgggctggcacctgactgtgcaataaccgtacatacccaggcagatacgtccagtcccgatccgttatttaatcctctaaaaactggcgtttgccaactggataacgcgaacgtgactgacgcgatcctcagcagggcaggagggtcaattgctgactttaccgggcatcggcaaacggcgtttcgcgaactggaacgggtgcttaattttccgcaatcaaacttgtgccttaaacgtgagaaacaggacgaaagctgttcattaacgcaggcattaccatcggaactcaaggtgagcgccgacaatgtctcattaaccggtgcggtaagcctcgcatcaatgctgacggagatatttctcctgcaacaagcacagggaatgccggagccggggtggggaaggatcaccgattcacaccagtggaacaccttgctaagtttgcataacgcgcaattttatttgctacaacgcacgccagaggttgcccgcagccgcgccaccccgttattagatttgatcaagacagcgttgacgccccatccaccgcaaaaacaggcgtatggtgtgacattacccacttcagtgctgtttatcgccggacacgatactaatctggcaaatctcggcggcgcactggagctcaactggacgcttcccggtcagccggataacacgccgccaggtggtgaactggtgtttgaacgctggcgtcggctaagcgataacagccagtggattcaggtttcgctggtcttccagactttacagcagatgcgtgataaaacgccgctgtcattaaatacgccgcccggagaggtgaaactgaccctggcaggatgtgaagagcgaaatgcgcagggcatgtgttcgttggcaggttttacgcaaatcgtgaatgaagcacgcataccggcgtgcagtttgtaa

SEQ ID NO: 61 - protein, 216 aa, Escherichia coli
MRCKGFLFDLDGTLVDSLPAVERAWSNWARRHGLAPEEVLAFIHGKQAITSLRHFMAGKSEADIAAEFTRLEHIEATETEGITALPGAIALLSHLNKAGIPWAIVTSGSMPVARARHKIAGLPAPEVFVTAERVKRGKPEPDAYLLGAQLLGLAPQECVVVEDAPAGVLSGLAAGCHVIAVNAPADTPRLNEVDLVLHSLEQITVTKQPNGDVIIQ

SEQ ID NO: 62 - DNA, 651 bp, Escherichia coli
  source 1..651: mol_type = genomic DNA
atgcggtgcaaaggttttctgtttgatcttgatggaacgctggtggattccctgcctgcggtagaacgggcgtggagcaactgggccagacgtcatgggttagcgccggaagaggtgctggctttcattcacggtaaacaggcgatcacctctctgcgccattttatggcgggcaaatccgaggctgatattgccgccgagtttacgcgtctggagcacatcgaggccacggaaaccgaaggtattaccgcgcttccgggggcaatcgccttactcagtcatttgaataaagcaggtattccgtgggccattgtgacttctggctccatgccggtagcgcgagcgcgccataaaatagctgggcttcccgcaccagaggtgtttgtaaccgctgagcgagtgaagcgcggaaaaccagaacctgatgcgtatctgttaggcgcgcagctgctggggcttgcgccgcaggagtgtgtggtggtggaagatgctcccgctggcgtgctttctggcctggcggcgggttgtcatgtcattgcggttaacgctccggcagataccccgcgcctgaatgaggtcgatttggtcctccacagtctggagcaaattactgtgaccaaacagccaaatggcgatgttattattcagtga

SEQ ID NO: 63 - protein, 336 aa, Escherichia coli
MRRELAIEFSRVTESAALAGYKWLGRGDKNTADGAAVNAMRIMLNQVNIDGTIVIGEGEIDEAPMLYIGEKVGTGRGDAVDIAVDPIEGTRMTAMGQANALAVLAVGDKGCFLNAPDMYMEKLIVGPGAKGTIDLNLPLADNLRNVAAALGKPLSELTVTILAKPRHDAVIAEMQQLGVRVFAIPDGDVAASILTCMPDSEVDVLYGIGGAPEGVVSAAVIRALDGDMNGRLLARHDVKGDNEENRRIGEQELARCKAMGIEAGKVLRLGDMARSDNVIFSATGITKGDLLEGISRKGNIATTETLLIRGKSRTIRRIQSIHYLDRKDPEMQVHIL

SEQ ID NO: 64 - DNA, 1011 bp, Escherichia coli
  source 1..1011: mol_type = genomic DNA
atgagacgagaacttgccatcgaattttcccgcgtcaccgaatcagcggcgctggctggctacaaatggttaggacgcggcgataaaaacaccgcggacggcgcggcggtaaacgccatgcgtattatgctcaaccaggtcaacattgacggcaccatcgtcattggtgaaggtgaaatcgacgaagcaccgatgctctacattggtgaaaaagtcggtactggtcgcggcgacgcggtagatattgctgttgatccgattgaaggcacgcgcatgacggcgatgggccaggctaacgcgctggcggtgctggcagtaggcgataaaggctgcttcctcaatgcgccggatatgtatatggagaagctgattgtcgggccgggagccaaaggcaccattgatctgaacctgccgctggcggataacctgcgcaatgtagcggcggcgctcggcaaaccgttgagcgaactgacggtaacgattctggctaaaccacgccacgatgccgttatcgctgaaatgcagcaactcggcgtacgcgtatttgctattccggacggcgacgttgcggcctcaattctcacctgtatgccagacagcgaagttgacgtgctgtacggtattggtggcgcgccggaaggcgtagtttctgcggcggtgatccgcgcattagatggcgacatgaacggtcgtctgctggcgcgtcatgacgtcaaaggcgacaacgaagagaatcgtcgcattggcgagcaggagctggcacgctgcaaagcgatgggcatcgaagccggtaaagtattgcgcctgggcgatatggcgcgcagcgataacgtcatcttctctgccaccggtattaccaaaggcgatctgctggaaggcattagccgcaaaggcaatatcgcgactaccgaaacgctgctgatccgcggcaagtcacgcaccattcgccgcattcagtccatccactatctggatcgcaaagacccggaaatgcaggtgcacatcctctga

SEQ ID NO: 65 - protein, 504 aa, Bifidobacterium adolescentis [sequence omitted]

SEQ ID NO: 66 - DNA, 1515 bp, Bifidobacterium adolescentis
  source 1..1515: mol_type = other DNA
atgaagaacaaagtgcagctgattacctatgcagatcgtttaggtgatggcaccattaaaagcatgaccgatattctgcgtacccgttttgatggtgtgtatgatggtgttcatatcctgccgttttttaccccgtttgatggcgcagatgcaggttttgatccgattgatcataccaaagtggatgaacgtttaggtagctgggatgatgttgcagaactgagcaaaacccataacattatggttgatgccattgtgaatcacatgagctgggaaagcaaacagtttcaggatgttctggcaaaaggtgaagaaagcgaatattatccgatgtttctgaccatgagcagcgtttttccgaatggtgcaaccgaagaagatctggcaggtatttatcgtccgcgtccgggtctgccgtttacacattacaaatttgcaggtaaaacccgtctggtttgggttagctttacaccgcagcaggttgatattgataccgatagcgataaaggttgggaatatctgatgagcatctttgatcagatggcagcaagccatgttagctatattcgtctggatgcagttggttatggtgcaaaagaagcaggcaccagctgttttatgaccccgaaaacctttaaactgattagccgtctgcgtgaagaaggtgttaaacgcggtctggaaattctgattgaagtgcacagctactacaagaaacaggttgaaattgccagcaaagttgatcgcgtttatgattttgcactgcctccgctgctgctgcatgcactgagcaccggtcatgttgaaccggttgcacattggacagatattcgtccgaataatgcagttaccgttctggatacccatgatggtattggtgttattgatattggtagcgatcagctggatcgtagcctgaaaggtctggttccggatgaagatgttgataatctggtgaataccattcatgccaatacacatggtgaaagccaggcagcaaccggtgcagcagccagcaatctggatctgtatcaggttaatagcacctattatagcgcactgggttgtaacgatcagcattatattgcagcacgtgccgttcagttttttctgcctggtgttccgcaggtttattatgttggtgcactggcaggcaaaaatgatatggaactgctgcgtaaaaccaataacggtcgtgatattaaccgccattattacagcaccgcagaaattgatgaaaatctgaaacgtccggttgtgaaagcactgaatgcactggccaaatttcgcaatgaactggatgcatttgatggcacatttagctataccaccgatgatgataccagcatttcatttacctggcgtggtgaaaccagccaggcgaccctgacctttgaaccgaaacgtggtctgggcgttgataataccacaccggtggcaatgctggaatgggaagatagtgccggtgatcatcgtagtgatgatctgattgcaaatccgcctgttgttgcataa

SEQ ID NO: 67 - protein, 984 aa, Clostridium thermocellum
MITKVTARNNKITPVELLNQKFGNKINLGNFADAVFTDAAFKNVAGIANLPMKAPVMQVLMENCIVSKYLKQFVPDRSVCFVEEGQKFYIVLEDGQKIEVPEDVNKALRATVSDVKHWAGYLTEDGEHVIDLLKPAPGPHFYVNLLIGNRLGFKRTLQTTPKSVVDRFGRGSFRSHAATQVLATRFDMRQEENGFPANRQFYLYEDGKQIFYSALIDDNIVEATCKHSCNRTVIKYKTACNLEITRTIFLVPHKKGFPLATELQRIEIKNASDKARNLSITYTGMFGTGAVHAIFEDVTYTNVIMQSAALYNDKGEFIGITPDYYPEEFKQDTRFVTMIVRNGDEKSFPQSFCTDYNDFVGTGTLEHPAGGCNLNNKLNRKGPGFFALGAPFTVEPGKTVIIDTFTGLSSSKDNENYSDAVMLRELDNLLRYFEKSESVEETLNEIINFHENYGKYFQFNTGNKLFDSGFNRNLAFQVLYQTFMSRSFGQTQKGYREIGFREIQDLFASMYYFINIGYQDFVKELLFEWTANVYKMGYANHNFYWVGKQPGLYSDDSLWLLQAYYRYIIYTKDTSVLNEEVPVADGNNEKRAVRETLKAIIQYSACISVGDHGLPLLDLADWNDCLKIDSNSIDGATKEKLYYEQLKKTNGKYGDRFMSDYSESVMNAFLLKLAIDHLAEIATLDNDTQLAQQMSELSKEVTDRIQKHAWKENFFARVLINRYKDGSYTYLGAKGDKLSADPNIDGVYFLNSFAWSVLSDVATDEQIAIMVDVIKKYLLTPYGLRLVTPADLNKIANDTATGHYFFGDRENGAVFKHASMMAVVALIKAAKKVKDNELAKEMARIAYFMIDLVLPYKNLENPFQVAGNPRICTQYINTDTGENIGPLLSGTATWLNLNLISLAGIEYTRDGISFNPILREEETQLNFTLKAPKCSYKFSITKPVGFARMESSEYELFVDGQKIDNTVIPMYTDEKEHIVTLKFK

SEQ ID NO: 68 - DNA, 2955 bp, Clostridium thermocellum
  source 1..2955: mol_type = genomic DNA
atgattactaaagtaacagcgagaaataataagataacacctgttgagttgttgaatcaaaagtttggaaacaagattaatctgggcaattttgcggatgctgtttttactgacgcggcgttcaaaaatgtggcaggcattgcaaatttgcctatgaaagcgccggtaatgcaggttcttatggaaaactgcattgtttcaaaatatctgaaacagtttgtacctgaccggtctgtttgttttgttgaagaaggacagaaattttacatagtacttgaagacggtcaaaaaattgaagtgcctgaggatgtaaacaaggctctcagggctacggtaagtgatgtaaagcattgggcaggttatttgacggaagacggggagcatgtaatcgaccttttaaaaccggctccgggtccgcatttttatgtgaatttgcttataggaaacaggcttggttttaaaaggacattgcagacaactccgaaaagtgtggttgacaggttcggaagaggttcgttccgttcccatgctgcaacccaggtgctggcaacgagatttgacatgcgccaggaggaaaacggttttcctgcgaacagacagttctatttgtatgaagacggcaaacagattttttattccgcattaattgatgacaacattgttgaggctacctgcaaacattcatgcaatcgtacggtaataaaatataagacggcatgtaatctggaaattacaagaaccatcttcctggtgcctcacaagaagggattccctcttgcaactgaattacagagaattgaaataaagaatgcgtcggacaaggcaaggaatttgtccattacatatacgggaatgtttggaacgggtgccgttcatgcgatatttgaggacgtaacatacacaaatgttatcatgcaaagtgccgccctttacaatgacaagggtgagtttatcggaataactcctgattattatcctgaagaatttaaacaggatacaagatttgtcacgatgattgtccgcaacggggacgagaaatcattcccgcagagtttctgcacggactacaacgactttgtaggcacaggaacattggagcatccggcaggcggatgtaatttgaacaacaagctgaaccgcaaaggtccgggattctttgccctgggtgcgccgtttacggttgaaccgggcaagacagtcataatagacactttcaccggtttgtcttcgagcaaggataatgaaaattacagcgatgcagtaatgctcagggaactggacaatttgctgcgctattttgaaaaaagcgaatctgtggaagaaacattgaatgaaattatcaacttccatgaaaattatggcaaatacttccagttcaataccggaaacaagctgtttgattccggatttaacaggaatttggcgttccaggtattgtatcagacatttatgtcccgttctttcggacaaacacagaaaggatatcgtgaaatcggattcagggaaattcaggacctgtttgcatccatgtactattttataaacataggatatcaggattttgtaaaggaattgttgtttgagtggacggcaaacgtatataaaatgggttatgcaaaccacaacttctattgggtgggcaaacagccgggactgtattccgatgacagcctgtggctcttgcaggcatattacagatatattatttatacaaaagatacttcggtattaaatgaggaagtaccggttgccgacggaaacaatgaaaagagggctgtaagagaaacgctgaaggctatcatccagtattccgcttgtatttctgtcggtgatcatggccttccgctgctggatcttgcagactggaatgactgcctgaagattgacagcaacagtatagacggtgcaaccaaagaaaagttgtactacgaacagttgaagaagacaaacggcaaatatggagatcgctttatgagcgattattcggaaagcgtgatgaatgctttcctcttgaagttggcaattgaccatttggctgaaattgcaactttggataatgacactcaactggcccaacaaatgagtgaattgtcaaaagaggttacagaccgcattcagaaacatgcctggaaagaaaacttctttgcccgtgttcttataaaccgttacaaagacggttcctatacttatttgggagcaaagggcgacaagctttccgctgatccgaacattgacggcgtgtacttcttaaacagttttgcatggtcggtgctgtccgatgttgcaaccgatgagcaaatagcaataatggtggatgtcatcaaaaaatatttgttaactccgtacggcttgcgtttggtaacacctgccgatttgaacaaaattgcaaatgatactgcaacagggcattacttctttggtgacagggaaaacggtgctgtcttcaaacatgcttcaatgatggcagttgttgcgcttatcaaggctgcaaagaaagtaaaagacaatgagcttgccaaagaaatggcaagaatagcgtactttatgatagacttggtactgccatacaagaaccttgaaaatccgttccaggttgcaggaaatccaaggatatgcactcaatatatcaatactgacacaggagaaaatattggacctttgttgagcgggacggcaacctggcttaacttgaatcttatttccctggcaggaatagagtacaccagggatggaatttccttcaatccgatacttcgggaagaggaaactcagttgaatttcactttgaaagcgccgaaatgctcatataagtttagtattacaaaaccggttggttttgctagaatggaaagttcggaatatgaactttttgttgatggacaaaagattgacaacactgtcattccaatgtatacggatgaaaaagaacatatagtgactcttaagtttaaataa

SEQ ID NO: 69 - protein, 811 aa, Clostridium thermocellum
MKFGFFDDANKEYVITVPRTPYPWINYLGTENFFSLISNTAGGYCFYRDARLRRITRYRYNNVPIDMGGRYFYIYDNGDFWSPGWSPVKRELESYECRHGLGYTKIAGKRNGIKAEVTFFVPLNYNGEVQKLILKNEGQDKKKITLFSFIEFCLWNAYDDMTNFQRNFSTGEVEIEGSVIYHKTEYRERRNHYAFYSVNAKISGFDSDRDSFIGLYNGFDAPQAVVNGKSNNSVADGWAPIASHSIEIELNPGEQKEYVFIIGYVENKDEEKWESKGVINKKKAYEMIEQFNTVEKVDKAFEELKSYWNALLSKYFLESHDEKLNRMVNIWNQYQCMVTFNMSRSASYFESGIGRGMGFRDSNQDLLGFVHQIPERARERLLDLAATQLEDGGAYHQYQPLTKKGNNEIGSNFNDDPLWLILATAAYIKETGDYSILKEQVPFNNDPSKADTMFEHLTRSFYHVVNNLGPHGLPLIGRADWNDCLNLNCFSTVPDESFQTTTSKDGKVAESVMIAGMFVFIGKDYVKLCEYMGLEEEARKAQQHIDAMKEAILKYGYDGEWFLRAYDDFGRKVGSKENEEGKIFIESQGFCVMAEIGLEDGKALKALDSVKKYLDTPYGLVLQNPAFTRYYIEYGEISTYPPGYKENAGIFCHNNAWIICAETVVGRGDMAFDYYRKIAPAYIEDVSDIHKLEPYVYAQMVAGKDAKRHGEAKNSWLTGTAAWNFVAISQWILGVKPDYDGLKIDPCIPKAWDGYKVTRYFRGSTYEITVKNPNHVSKGVAKITVDGNEISGNILPVFNDGKTHKVEVIMG

SEQ ID NO: 70 - DNA, 2436 bp, Clostridium thermocellum
  source 1..2436: mol_type = genomic DNA
atgaagttcggtttttttgatgatgcaaacaaagagtacgttattaccgtgcccaggacaccgtatccgtggataaactacctgggtacagagaatttcttctcactcatttcgaataccgcaggcggatattgcttttacagggatgcaaggcttagacgtataacaagatacagatacaacaatgttcctattgacatgggaggacgttatttctacatatatgacaacggtgatttctggtcgccgggatggtctccggtaaaaagggagcttgaaagctatgaatgcagacatggactgggatatacaaaaattgccggtaaaagaaacggaataaaagcggaggtcactttcttcgttccgttaaactacaatggtgaagtccaaaagcttatattgaagaatgaaggacaggacaaaaagaaaataactctcttctcttttattgagttctgcttgtggaatgcttatgatgatatgaccaacttccagagaaacttcagcaccggtgaagttgagattgaaggctcggttatctatcacaagacagagtacagagagcgcagaaaccattacgcattctattctgtaaatgcaaaaatcagcggatttgacagtgacagagacagcttcataggactttacaacggttttgacgctcctcaggctgtagtgaacggcaagtcaaacaattccgttgcggacggatgggcaccgattgcgtcccacagcattgaaattgaattgaatcccggggagcaaaaggaatatgtatttattataggttatgtggagaacaaagatgaagaaaaatgggagtcaaaaggtgtcatcaacaagaaaaaagcttatgaaatgatagagcagttcaacactgttgaaaaggttgacaaagcatttgaagaactcaagagctattggaatgctcttctttcaaaatactttcttgaaagccacgatgaaaaactcaaccgtatggttaatatatggaatcagtaccagtgtatggttacattcaacatgtcaagaagcgcttcatactttgaatccggtatcggaagaggtatgggtttcagagattcaaaccaggacttgctgggatttgtacaccagatacccgaaagagcaagagaaaggcttcttgacctggctgcaactcagcttgaagatggcggtgcgtaccatcagtatcagcctcttaccaaaaaaggtaacaatgaaatcggaagcaacttcaacgatgacccgttgtggctgattcttgcaactgctgcatatattaaggaaaccggtgattattcaatactgaaggagcaagttccgttcaacaatgatccgtccaaagccgacaccatgtttgaacatttgacccgttccttctaccatgtggtaaacaaccttggacctcacggattgccgcttataggtagggcggactggaatgactgccttaacttaaactgcttctccaccgttccggatgagtcgttccagaccacaacaagcaaagacggaaaagtggcagagtcagttatgattgccggaatgtttgtgttcatcggaaaagactatgtgaagctttgcgaatacatgggccttgaagaggaagccaggaaagctcagcagcatattgacgcaatgaaggaagcaattctcaaatacggttatgacggtgagtggttcttaagagcttacgacgactttggaagaaaagtcggaagcaaagaaaacgaagagggtaagattttcattgagtctcagggattctgtgtaatggctgaaatcgggcttgaagacggcaaggctttgaaggctctggattctgtcaagaaatatcttgacactccatatggtcttgtacttcaaaatcccgcgtttacaagatactatattgagtacggagaaatttcaacatatccaccgggatacaaagaaaatgccggtatattctgccacaacaatgcatggataatctgtgctgaaacggttgtcggaagaggagacatggcgtttgattactatagaaaaatagcacctgcttatattgaagatgtaagtgacatccacaagcttgagccttatgtttatgcacagatggttgccggaaaagacgcaaaacgccatggagaagctaagaactcatggctgaccggtactgcggcgtggaactttgtggcgatttcacagtggatactgggtgtaaaacctgactatgacggattgaagattgatccatgcatacccaaggcatgggacggatacaaagttaccagatatttcagaggctcaacttatgaaatcactgtgaagaatccgaaccatgtatcaaaaggtgtggctaaaattactgttgacggcaatgaaatcagcggaaatattcttccggtgttcaatgacggaaagactcacaaagttgaagtaattatgggataa